European Patent Specification EP 3 781 586 B1, published April 17, 2024. Title: Process for the manufacture of icatibant. Applicant: Fresenius Kabi iPSUM Srl. The sequence listing filed with the application follows.

SEQUENCE LISTING (2 sequences)

SEQ ID NO: 1 - protein, 5 aa, Artificial Sequence
  equivalent of a fragment of icatibant (amino acid moieties 1-5 of icatibant) containing only L-amino acid moieties
  Xaa (4)..(4): 4-hydroxyproline
RRPXG

SEQ ID NO: 2 - protein, 4 aa, Artificial Sequence
  fragment of icatibant (amino acid moieties 2-5 of icatibant)
  Xaa (3)..(3): 4-hydroxyproline
RPXG